European Patent Specification EP 3 811 972 B1, published January 11, 2023. Title: Combination Therapy for Treatment of Coronary Artery Disease. Applicant: The Board of Trustees of the Leland Stanford Junior University. The sequence listing filed with the application follows.

SEQUENCE LISTING (6 sequences)

SEQ ID NO: 1 - DNA, 24 bp, Homo sapiens
tggcaggggcgggcccaagggctg

SEQ ID NO: 2 - DNA, 24 bp, Homo sapiens
cagcccttgggcccgcccctgcca

SEQ ID NO: 3 - DNA, 19 bp, Homo sapiens
aggtccaatggaaaaagac

SEQ ID NO: 4 - DNA, 20 bp, Homo sapiens
cagaaactgctccttgaagt

SEQ ID NO: 5 - DNA, 20 bp, Homo sapiens
ccggaagcacttctcctaga

SEQ ID NO: 6 - DNA, 20 bp, Homo sapiens
aagagagagcggaagtgacg